European Patent Application EP 4 509 604 A1, published February 19, 2025. Title: 新規リパーゼ. Applicant: 花王株式会社. The sequence listing filed with the application follows.

SEQUENCE LISTING (50 sequences)

SEQ ID NO: 1 - DNA, 876 bp, synthetic construct
  source 1..876: mol_type = other DNA; note = Cedecea sp.-derived sequence
atgtctacatcactgaaatatccgattgtccttgttcatggcctgcttggatttgataaaattggcggaatctacccgtacttttacggaatcaaagaagcgctggaaaaagcaggcgcgaaagtgtatatcgcaacattaagcgcgctgaattctaacgaaatgagaggagaacaattactggaatttgtgcgcaaagtccaggctgaaacaggcgcagcgaaagttaatcttattggccattctcaaggaccgttagcttgcagatatgtggctgccacacatccggatctgatcgcctcagttacaagcgtgaatggcgtcaaccatggatcagaagttgctgatcttgtgagactggcccttaaaccgggacgcttaccggaatcaattgcaaatgcagcgctgagcgcgtttggccaacttttatctgctttagctggagaaccgagactgcctcagtcaggcgtggatgcacttgatgcgttaacaagcgaaggagtcgctgcctttaacaaaaaatatccgcaaggattacctgcagaatggggcggacagggaaaagaactggataacggagtctactactacagctggtctggaattatcgattataacccgctgcatcaaggcatgaataacctggatccgcttcatgttgctatgcttgcctttagcatcctgtttacaaacgaaagatttcagaacgatggcctggtgggacgctattcaagccatcttggcaaagtcattggatctgattattcaatggatcatgttgatgcgatcaatcaactggctggagttgtggccaataacacagatccggtcaaactttatgttgatcatttagcaagactgcaggcgaaaggctta

SEQ ID NO: 2 - protein, 292 aa, Cedecea sp.
MSTSLKYPIVLVHGLLGFDKIGGIYPYFYGIKEALEKAGAKVYIATLSALNSNEMRGEQLLEFVRKVQAETGAAKVNLIGHSQGPLACRYVAATHPDLIASVTSVNGVNHGSEVADLVRLALKPGRLPESIANAALSAFGQLLSALAGEPRLPQSGVDALDALTSEGVAAFNKKYPQGLPAEWGGQGKELDNGVYYYSWSGIIDYNPLHQGMNNLDPLHVAMLAFSILFTNERFQNDGLVGRYSSHLGKVIGSDYSMDHVDAINQLAGVVANNTDPVKLYVDHLARLQAKGL

SEQ ID NO: 3 - DNA, 861 bp, synthetic construct
  source 1..861: mol_type = other DNA; note = Proteus vulgaris-derived sequence
atgagtacgacttatccgattgttttggtacacggactctccggctttgatgacatagtcggctacccttatttttacggaatcgcagacgcactggagaaggacggacataaagtgttcacggcctcgctttcggcttttaacagcaatgaagtccgcggagagcagctttgggaatttgttcaaaaaattctgaaggaaacaaaagcgaagaaagttaacctgatcggccattcacaaggaccgcttgcctgcaggtacgtggcagcaaagcatgcaaaaagcatagcatctgttacatctgtcaacggagtgaatcacggcagtgaaattgcggatttggtgcgccggatcatgagaaaagacagcgtaccagagtacattgctgatgcggtcatgaaagcgatcggtaccatcattagcaccttttccgggaaccgaggaaatccgcaggatgccattgccgcgttagaggctttaactacagaaaatgtgatggaattcaataaaaaatatcctcaaggtcttccagccattcgcggcggcgaaggcaaggaagtggtcaatggtgttcattattattcatttggttcttatattcaaggcctcatcgcgggagaaaaagggaatcttttggatcccacacacgctgcgatgcgtgtattgtcagcgtttttctctgaaagagaaaacgacggcttagtaggcagaacgagcatgcggttaggaaaactgattaaagatgattatgcagaggatcatttagatatggtgaaccaggttgctgggctcgtcgggcgtggggaagatatcattgcaatatatacaaatcatgccaatttcctggcttcaaaaaagcta

SEQ ID NO: 4 - protein, 287 aa, Proteus vulgaris
MSTTYPIVLVHGLSGFDDIVGYPYFYGIADALEKDGHKVFTASLSAFNSNEVRGEQLWEFVQKILKETKAKKVNLIGHSQGPLACRYVAAKHAKSIASVTSVNGVNHGSEIADLVRRIMRKDSVPEYIADAVMKAIGTIISTFSGNRGNPQDAIAALEALTTENVMEFNKKYPQGLPAIRGGEGKEVVNGVHYYSFGSYIQGLIAGEKGNLLDPTHAAMRVLSAFFSERENDGLVGRTSMRLGKLIKDDYAEDHLDMVNQVAGLVGRGEDIIAIYTNHANFLASKKL

SEQ ID NO: 5 - DNA, 870 bp, synthetic construct
  source 1..870: mol_type = other DNA; note = Pseudomonas frederiksbergensis-derived sequence
atgaatatggacgcgtcaacgcaatatccgatagtgcttgttcacggtttgtttggcttcgatacaatcggcggatacccttatttttttgaaatcaaagaagcgcttgaaagggcgggagcaaaagtgtacgctgtcaatattccagcggttaacggcaatgaagagcggggagaaaaactattggagcatgtgaaccgcattcttcgcgaaacaggcgccgccaaggtcaacctgatcggacattcacaaggcccgctggcagcccgatacgtggcagctctgcatccgcaaaaagtagccagtgtcactagtgtgagctgtcccaatcatggatcggaaattgctgatcagcttcataaagcgctgacgcctggcgagctgccagaagcagttgttctggcattattcgccgctgtcggcattttcatctccctaatatccgggcatcctgaaaatccgcaggacgcgcgtgctgcctttgcatcactcacctctgaaggtcttgcggcttttaacaaaaagtatccccagggggttccgaaacattggggtggcgacgggaatgagattgaaaacggagtttattattactcttggtcaggtattgttcagaattttcaatccttacagccactggatccgagccacttaaactgcattgtgctcagtaagctgttttataaagagaaacacgcgaatgacggacttgtcggacaaaacagctctcatttggggaaagtaatcagatctgattatccgatggatcattttgatgctgtaaatcaaatggcagggattacaagctggaatgtctcgcctgtacacctctatttggaacacgcagcaagattaaaggataaaggctta

SEQ ID NO: 6 - protein, 290 aa, Pseudomonas frederiksbergensis
MNMDASTQYPIVLVHGLFGFDTIGGYPYFFEIKEALERAGAKVYAVNIPAVNGNEERGEKLLEHVNRILRETGAAKVNLIGHSQGPLAARYVAALHPQKVASVTSVSCPNHGSEIADQLHKALTPGELPEAVVLALFAAVGIFISLISGHPENPQDARAAFASLTSEGLAAFNKKYPQGVPKHWGGDGNEIENGVYYYSWSGIVQNFQSLQPLDPSHLNCIVLSKLFYKEKHANDGLVGQNSSHLGKVIRSDYPMDHFDAVNQMAGITSWNVSPVHLYLEHAARLKDKGL

SEQ ID NO: 7 - DNA, 882 bp, synthetic construct
  source 1..882: mol_type = other DNA; note = Enterobacillus tribolii-derived sequence
atgaaaaaagcaactacgcttaaatatccgattatcttggtgcacggactttttggttttgacaaaatcgctggcgtttatccttattttttcggtgtaaaagaagctcttgaaaaagcgggggcggaagtgtatgtcgcatcactgtcggcagtaaattcaaacgaagttcgcggtgagcagctcatggactttgtcaatgaggtgctggcaaataccggtgcaaagaaggtgaacttgatcggccactctcaaggcccgcttgcctgccgttacgtggctgcattacgccctgatattgttgcttctgtgacaagcgttcatggcgtcaacttcggcagcgagttagccgatgtggtccgtcaggccttgattccagggaggttgcctgaagcgatagctcatgcggtagtcacaacatttggagatttcttatcgctaatttcaggaaagccgatgcttgcgcaggatgcaaaagccgccttagacgcccttacctcagaaggaatcgcagaatttaatgcgaagtacccgcaagggctgccatctgaatggggaggagaaggcgatgaatatgtaaacggcgtatattattacagctggggcggagttttaaaatacaatatctttgatcagctgttgaacaatctggatcccacacatattgcgatgagtgctctttccattttctttaacaaagagcggggacaaaatgacggcgttgtcggtagatactctatgcatttaggaaaagttatacgatctgattattcaatggatcacctcgacgctgtaaatcaaacggcaggggttgtcacgactagtgtcaatccggtgaagctgtatgttgatcatttgtatcttctgagaagcaaaggcctc

SEQ ID NO: 8 - protein, 294 aa, Enterobacillus tribolii
MKKATTLKYPIILVHGLFGFDKIAGVYPYFFGVKEALEKAGAEVYVASLSAVNSNEVRGEQLMDFVNEVLANTGAKKVNLIGHSQGPLACRYVAALRPDIVASVTSVHGVNFGSELADVVRQALIPGRLPEAIAHAVVTTFGDFLSLISGKPMLAQDAKAALDALTSEGIAEFNAKYPQGLPSEWGGEGDEYVNGVYYYSWGGVLKYNIFDQLLNNLDPTHIAMSALSIFFNKERGQNDGVVGRYSMHLGKVIRSDYSMDHLDAVNQTAGVVTTSVNPVKLYVDHLYLLRSKGL

SEQ ID NO: 9 - DNA, 882 bp, synthetic construct
  source 1..882: mol_type = other DNA; note = Escherichia sp.-derived sequence
atgaagattcagacgcaattaaattaccctgtcgtgcttgtccacggcttgttcggttttgataaaattgcaggggtttatccgtatttttacggcatcaaagatgccttggaagaagctggggccaccgtgttcatcgcttctatttcagcagtaaatgacaatgagcttcggggagagcagctgcttgcatatatcaatgatgtgctgaaaaaaacaggaaaagagaaggttaacctcatcggccattcacaggggcctttggcttgccgctatgtggctgcaacacaccccacattagttgcctctgtcacttctgtaaacggtgtgaatttcggctcagagttcgcggacctcgttagatctgcgctcattccgggtgaaatccctgaagtcattgccaacagtatacttgacgtttttgcgaagctgctgacggccatctccggaaatccggattttccgcaggattcgatagctgcgctggatgcgctaacaacggaaggggtagcaaaatttaacgaaaaatatcctcaaggactcccgattgtacgcggcggtgaaggcaaagaatttgacaacggtgtatattattacagctggagcggcattatagacagcaatatcctgcatcaaggcatgaataactttgatccatctcatattgcgatgctcgcttgtagcatgctgtttgaaaatgaatatcatgaaaacgacggacttgtcggccgttatgcgtcccacttaggaaaggttatcagaagcgattattcgcttgatcatttggatgcaattaatcaaattgcaggagtgttgccacgatacagtgattcaatctccatttaccttgagcatttagagaggttaaaatcaaaaggatta

SEQ ID NO: 10 - protein, 294 aa, Escherichia sp.
MKIQTQLNYPVVLVHGLFGFDKIAGVYPYFYGIKDALEEAGATVFIASISAVNDNELRGEQLLAYINDVLKKTGKEKVNLIGHSQGPLACRYVAATHPTLVASVTSVNGVNFGSEFADLVRSALIPGEIPEVIANSILDVFAKLLTAISGNPDFPQDSIAALDALTTEGVAKFNEKYPQGLPIVRGGEGKEFDNGVYYYSWSGIIDSNILHQGMNNFDPSHIAMLACSMLFENEYHENDGLVGRYASHLGKVIRSDYSLDHLDAINQIAGVLPRYSDSISIYLEHLERLKSKGL

SEQ ID NO: 11 - DNA, 882 bp, synthetic construct
  source 1..882: mol_type = other DNA; note = Yersinia enterocolitica-derived sequence
atgagcacgaacagcactttaaaatacccggttgtgttagttcacggcctgcttggttttgataagatcgccggtgtttatccatatttttacggcgttgaagaacctttgaaaaaagcgggcgcacaggtgtttgtcgcaaccatctccgctacaaactcaaatgaagtaagaggcgaacagcttttgaagtttgtgaaagaagtcatggcaaaaacaggagccaagaaagtgaacttgatcggccacagccaaggcccgctagcttgccgatatgtggcggcgactcatccggagcttattgcatctgtaacgtcagtaaacggggtcaatcacgggagtgagattgctgaccttgtcagatcggctttggtcccaggatcactccccgagcatattgtgaatacaattatgagtgctttcggagtattcgtttctcttttatccggaaaaccgttcctgcctcaggattttatggaaagcatcgacgcgctgaccacagaaaatgtcgcgaaatttaacacgaaatatccgcagggtcttcctgaaacgtgggggggcgaggggaaagaatttgacaatggcgtatattattacagctggggaggtgtccttggctataacccgctcattgaaggcttaaataatctggatccactccatcattctctcgtggccttatcgctgctgttcacaaaagaacgcaaccaaaatgacgggttagtcggtcggtactccatgcatttaggtaaagtcatacgttcagattatcaacttgatcatgttgatgccatcaatcaaacagcaggaatggtttcaaaggatatagatcctgttcaattatttgttaatcagattgaattgctgaagtctaaaggactg

SEQ ID NO: 12 - protein, 294 aa, Yersinia enterocolitica
MSTNSTLKYPVVLVHGLLGFDKIAGVYPYFYGVEEPLKKAGAQVFVATISATNSNEVRGEQLLKFVKEVMAKTGAKKVNLIGHSQGPLACRYVAATHPELIASVTSVNGVNHGSEIADLVRSALVPGSLPEHIVNTIMSAFGVFVSLLSGKPFLPQDFMESIDALTTENVAKFNTKYPQGLPETWGGEGKEFDNGVYYYSWGGVLGYNPLIEGLNNLDPLHHSLVALSLLFTKERNQNDGLVGRYSMHLGKVIRSDYQLDHVDAINQTAGMVSKDIDPVQLFVNQIELLKSKGL

SEQ ID NO: 13 - DNA, 879 bp, synthetic construct
  source 1..879: mol_type = other DNA; note = AncLip1
atgaatacagaagcgacaacaaaatacccaattgtgcttgttcatggtctattcggctttgataagatcgccggctacccttattttttcggtattaaggaggcacttgagaaggcgggagcaaaagtatttacgccttcaatatccgcagtcaactcaaatgaagtgaggggggagcagctgttagaacaggttcagcgaattctgaaaaaaacaggggctcaaaaagtgaatttaatcggtcacagccaagggccgctggcctgccgctatgtagctgcgatgcatccggaactggtcgcatctgtgacaagtgtctccggaccgaatcatgggagtgaaatcgcagatcagcttcggaaagcgctgaccccaggcgagttgcccgaggctgttgcatcaaccctgatgaacgcctttggaaactttatttctctcctttctggacaccctcagctcccgcaggatgctgtcgctgcattagatgccttgacgactgaaggcgttgctgaatttaacagaaaatatccacaaggccttcctgaaacatggggcggagaaggaaaagaaattgaaaacggagtatactattattcgtggagcggcattatcaaaggatcgattttggaccaaggattaaatacgcttgatccgcttcacttagcatgtcgcgcgctctcaaagctgttcactaaggaaaaaaatcaaaatgacggtctcgtaggaagatactccagccatttaggcaaagtcatccgttctgattatccgatggatcatttggatgccgtgaaccaaacggcgggtgtcgtttcaactaatgtagacccggtgaagctttatgttgaccatgcggctttattgaaaagcaaaggcttg

SEQ ID NO: 14 - protein, 293 aa, synthetic construct
  source 1..293: note = AncLip1
MNTEATTKYPIVLVHGLFGFDKIAGYPYFFGIKEALEKAGAKVFTPSISAVNSNEVRGEQLLEQVQRILKKTGAQKVNLIGHSQGPLACRYVAAMHPELVASVTSVSGPNHGSEIADQLRKALTPGELPEAVASTLMNAFGNFISLLSGHPQLPQDAVAALDALTTEGVAEFNRKYPQGLPETWGGEGKEIENGVYYYSWSGIIKGSILDQGLNTLDPLHLACRALSKLFTKEKNQNDGLVGRYSSHLGKVIRSDYPMDHLDAVNQTAGVVSTNVDPVKLYVDHAALLKSKGL

SEQ ID NO: 15 - DNA, 864 bp, synthetic construct
  source 1..864: mol_type = other DNA; note = AncLip2
atgagcacgaaatatccgattgtgttagtacacggtttattcggttttgataaaatcgccggctatccttatttttttggaattaaagatgcactgaaaaaggcagggcataaagtatttacagcctccctctcggctgttaacagcaatgaagtgagaggcgagcagctgtgggaatttgtacaggaaatcctgaagaagacgggagctaaaaaagtgaacttgatcggtcacagtcaggggccccttgcatgccgctatgtcgcggccatgcatcctgaatcagtagcttctgttacttctgttaacggagtaaatcacggctcagaaattgcggacctcgtccggaaggtgctgacgccgggcagccttccggaagcagttgcgaacacagtcatgaatgccttcggcacgtttatttctctactatccggacatccgcaaaaacctcaggatgccgtcgctgcgcttgaggcgttaaccacagaaggcgtaaccgagtttaataaaaaatacccacaagggcttccaaaaacatggggaggagaaggaaaagagatcgtgaacggcgttcattattactcttttgggtcgttcattaaaggaagcatattagatcaaggcctgaatatgttggacccgactcatttggcaatgagagctttgagtaaatttttcacaaaagaaaaacaaaatgacggattagtcggccgttattcaatgaggctgggtaagctgatacgagatgattacagcatggatcatcttgatatggtgaatcaagtggcgggtgttgtttcaacaaacgttgacatcgtcaagatttatgtgaatcatgcaaagcttttagcatcaaaaggcctc

SEQ ID NO: 16 - protein, 288 aa, synthetic construct
  source 1..288: note = AncLip2
MSTKYPIVLVHGLFGFDKIAGYPYFFGIKDALKKAGHKVFTASLSAVNSNEVRGEQLWEFVQEILKKTGAKKVNLIGHSQGPLACRYVAAMHPESVASVTSVNGVNHGSEIADLVRKVLTPGSLPEAVANTVMNAFGTFISLLSGHPQKPQDAVAALEALTTEGVTEFNKKYPQGLPKTWGGEGKEIVNGVHYYSFGSFIKGSILDQGLNMLDPTHLAMRALSKFFTKEKQNDGLVGRYSMRLGKLIRDDYSMDHLDMVNQVAGVVSTNVDIVKIYVNHAKLLASKGL

SEQ ID NO: 17 - DNA, 882 bp, synthetic construct
  source 1..882: mol_type = other DNA; note = AncLip3
atgaaaacgtccacgacgctgaagtatccgattgttctcgttcatggtctctttggctttgataaaatagctgggatttatccttatttcttcgggattaaagaggcgctggagaaggcaggtgcaaaagtgtttaccgcatccatttcggctgtaaacagcaatgaagtccgaggagaacagcttcttgagtttgtcaaagaggtacttgctaaaacaggagcaaaaaaggtgaatctgatcggtcacagtcaaggcccactggcctgccgctatgtcgcggccatgcatcctgagttggttgcctcagttacctctgttaacggtgtcaatcatggcagtgaaatcgcagatcttgtcagaaaagctttaacaccaggctctcttccggaagcgatcgctaatacagtcatgaatgcgttcggaaattttctttcactgatttcggggcatccgcagctgccgcaagatgctgttgcggccttagatgcactaacaactgaaggtgtagcagaattcaacgctaagtaccctcagggccttcctgaaacatggggaggcgaaggaaaagaatttgaaaacggcgtttactattatagctggggcggaatcatcaaatacaacattttagaccaaggattgaacaaccttgatccgcttcacattgcaatgagagcgttatctttgttttttacaaaagaacggaatcaaaatgatgggctcgtgggcaggtacagcatgcacttgggtaaggtcatacgttctgattattcaatggatcatctggacgcggtgaatcagactgccggagtggtcagcacgaatgtggaccccgtaaagctgtatgtagaccatgtggccctcttgaaatcaaaaggatta

SEQ ID NO: 18 - protein, 294 aa, synthetic construct
  source 1..294: note = AncLip3
MKTSTTLKYPIVLVHGLFGFDKIAGIYPYFFGIKEALEKAGAKVFTASISAVNSNEVRGEQLLEFVKEVLAKTGAKKVNLIGHSQGPLACRYVAAMHPELVASVTSVNGVNHGSEIADLVRKALTPGSLPEAIANTVMNAFGNFLSLISGHPQLPQDAVAALDALTTEGVAEFNAKYPQGLPETWGGEGKEFENGVYYYSWGGIIKYNILDQGLNNLDPLHIAMRALSLFFTKERNQNDGLVGRYSMHLGKVIRSDYSMDHLDAVNQTAGVVSTNVDPVKLYVDHVALLKSKGL

SEQ ID NO: 19 - DNA, 882 bp, synthetic construct
  source 1..882: mol_type = other DNA; note = AncLip4
atgagcacttcaactacgctgaagtacccgattgttcttgtccacggtttgttcggatttgataaaatcgcgggtatttatccttatttttacggcatcaaggaggcgttagaaaaagccggcgcaaccgtgttcacggcatcaatcagcgctgtaaattctaatgaggtacgcggagaacagttgcttgaatttgtgaaagaagtgcttgcaaaaacaggcgccaaaaaagtgaacctcattggacattctcaaggcccgcttgcctgccgttatgtggccgcgatgcatccagagctcgtggcttctgttacatccgtcaacggtgtcaatcatgggtccgaaatcgctgatctcgtaagatcggcgctgacaccgggatcgctgcctgaagcaattgcgaacaccgtcatgaatgcgttcggtaactttttgagcctaataagtgggcatccacagctgcctcaggactcagtagcagcacttgacgctttaacaactgaaggagttgctaaatttaatgccaaatatccccaggggctgccagaaacatggggcggcgaaggcaaggagtttgaaaatggggtttattattacagctgggggggcataattaactataatccgctggatcaaggattaaacaatttagaccctcttcatattgcaatggttgcgttgtctctgttatttacaaaagagagaaaccaaaatgatggactagtcggcaggtattcaatgcacttgggaaaagtcattcggagtgactacagcatggatcaccttgatgccatcaatcaaacggcaggtgttgtatcctctgatgtggatccggttaagctgtatgtcgaccatgttgctttactaaagtcaaaaggattg

SEQ ID NO: 20 - protein, 294 aa, synthetic construct
  source 1..294: note = AncLip4
MSTSTTLKYPIVLVHGLFGFDKIAGIYPYFYGIKEALEKAGATVFTASISAVNSNEVRGEQLLEFVKEVLAKTGAKKVNLIGHSQGPLACRYVAAMHPELVASVTSVNGVNHGSEIADLVRSALTPGSLPEAIANTVMNAFGNFLSLISGHPQLPQDSVAALDALTTEGVAKFNAKYPQGLPETWGGEGKEFENGVYYYSWGGIINYNPLDQGLNNLDPLHIAMVALSLLFTKERNQNDGLVGRYSMHLGKVIRSDYSMDHLDAINQTAGVVSSDVDPVKLYVDHVALLKSKGL

SEQ ID NO: 21 - DNA, 882 bp, synthetic construct
  source 1..882: mol_type = other DNA; note = AncLip5
atgtcaatcaacagcaccctcaaataccccgttgtattagtgcacggcctgctcggttttgacaaaatcgcagggatatacccgtatttttatggcattgaagaaccactgaaaaaagcgggtgcggatgtcttcgtggctacaatctctgcgacaaattcaaatgaagtcagaggtgaacagctgttgaagttcgtaaaagaggtcatggcaaaaacaggagccaagaaagtaaatctaatcgggcactctcaagggccgcttgcctgccggtacgtagctgcaactcatccggaattgattgcctctgttacttcagtcaatggggttaatcacggaagtgagatagctgatcttgtacgatcggcgctgacgccaggtagtttacctgagcagattgtaaacacgattatgtcggctttcggcgtgttcgtgtcactgctgtccggcaaaccgtttttaccgcaggactttatggaaagcattgatgctctcacgacagaaaatgtggcgaaatttaatacaaaatatcctcagggactgcctgaaacatggggtggagaaggaaaagaatttgataacggtgtttattattacagctggggcggcattttaggatacaacccacttacggaaggccttaacaaccttgatccgctgcatcattcaatggttgccttatcgcttttgtttacaaaggagagaaaccaaaatgacggccttgtcggacgctatagcatgcatttgggaaaggtcatccgttctgattataaattagatcatgtcgacgcaatcaatcaaaccgcaggaatggtgtcctccgacgttgatcctgttcaattgtatgtgaatcatattgagcttttaaaaagcaagggcttg

SEQ ID NO: 22 - protein, 294 aa, synthetic construct
  source 1..294: note = AncLip5
MSINSTLKYPVVLVHGLLGFDKIAGIYPYFYGIEEPLKKAGADVFVATISATNSNEVRGEQLLKFVKEVMAKTGAKKVNLIGHSQGPLACRYVAATHPELIASVTSVNGVNHGSEIADLVRSALTPGSLPEQIVNTIMSAFGVFVSLLSGKPFLPQDFMESIDALTTENVAKFNTKYPQGLPETWGGEGKEFDNGVYYYSWGGILGYNPLTEGLNNLDPLHHSMVALSLLFTKERNQNDGLVGRYSMHLGKVIRSDYKLDHVDAINQTAGMVSSDVDPVQLYVNHIELLKSKGL

SEQ ID NO: 23 - DNA, 882 bp, synthetic construct
  source 1..882: mol_type = other DNA; note = AncLip6
atgtcaacatctaccactttaaaatatccgattgttctagtccatggattattcggatttgataaaattgccgggatctatccatatttttacggaataaaggaagcacttgaaaaagctggagccacagtatttaccgcatcaataagtgctgttaacagcaatgaagtgagaggtgaacagcttttggagtttgtaaaagaggtgctggccaaaacaggcgcggaaaaggtaaacctcatcggccattcacaaggacctctggcttgccgctatgtagcggcaacgcacccagagctggtggctagcgtcacgtcagtcaatggcgtgaatcacggcagtgaaattgctgatcttgttcgttccgcattgaaaccgggttcgctccctgaagcaattgccaacacggtgatgaatgctttcggacaatttttatctgcgatttcagggcatccgcagctgccccaagactcggttgcggcccttgatgcgctgacgactgaaggagttgccaaatttaacgcgaagtaccctcagggcctgccggccacatggggcggagagggcaaggaatttgacaacggcgtgtattactatagctggtccggaatcatcaactacaatccgctcaatcaagggttaaataatctggaccctttgcatattgcaatggttgcccttagcctattgtttacaaaagaacggttccaaaacgacggtttagtaggtagatactccagccatctggggaaagtcattaggtcagattattctatggatcaccttgatgctatcaatcagacagcgggtgtcgtgtcctctgacgctgatccggttaagttgtatgtcgatcatgtcgcacgattgaaatctaaaggcctt

SEQ ID NO: 24 - protein, 294 aa, synthetic construct
  source 1..294: note = AncLip6
MSTSTTLKYPIVLVHGLFGFDKIAGIYPYFYGIKEALEKAGATVFTASISAVNSNEVRGEQLLEFVKEVLAKTGAEKVNLIGHSQGPLACRYVAATHPELVASVTSVNGVNHGSEIADLVRSALKPGSLPEAIANTVMNAFGQFLSAISGHPQLPQDSVAALDALTTEGVAKFNAKYPQGLPATWGGEGKEFDNGVYYYSWSGIINYNPLNQGLNNLDPLHIAMVALSLLFTKERFQNDGLVGRYSSHLGKVIRSDYSMDHLDAINQTAGVVSSDADPVKLYVDHVARLKSKGL

SEQ ID NO: 25 - DNA, 882 bp, synthetic construct
  source 1..882: mol_type = other DNA; note = AncLip7
atgagtacaagcacgacgctgaagtatccgattattttagttcatggattttccggctttgataaaatcgcaggcatttatccttatttttatggtattcagcaggcgctcgagaaagcaggtgcaacagtattcaccgcatctatttctgcggaaaattcaaatgaagtgcgaggtgaacagcttcttgaatttgtcaaacaagtgatcgccttgaccggcgctgaaaaagttaatctgatcggacattcacaagggccgctggcttgccgctatgtagctgctatgcatccggagctggttgcctcggtaacgtctgtgaacggcgtcaacttcggttctgaaatcgctgacttagtacggctcgcagtgaagcccggaagcctgccagaagcgattgcatccacggtcatgaatgccttcggcagctttttatccctcattacagggcatccttcgctgcctcaggacagtgtggcggccttagatgctctcacttcagaaggagtcgcaaaatttaatgcgaaatacccgcaagggcttccgtcaacatggggcggagaaggcaaggagtttgaaaacggggtttattattacagctggggaggaatcataaactacaaccctcttgatcaaggcttaaataacttagacccacttcacactgcgatggttgcgctttctctgttgttcacaaaagagagatttcaaaatgatggacttgtcgggcgttacagcatgcacttgggaaaagtgataaggagcgattattcaatggatcatttggacgccattaatcaaacagctggtgttgtcacttctgatgccgatccggttcagctgtttgttgaccacgtggcgagattgaagtcaaaaggcctt

SEQ ID NO: 26 - protein, 294 aa, synthetic construct
  source 1..294: note = AncLip7
MSTSTTLKYPIILVHGFSGFDKIAGIYPYFYGIQQALEKAGATVFTASISAENSNEVRGEQLLEFVKQVIALTGAEKVNLIGHSQGPLACRYVAAMHPELVASVTSVNGVNFGSEIADLVRLAVKPGSLPEAIASTVMNAFGSFLSLITGHPSLPQDSVAALDALTSEGVAKFNAKYPQGLPSTWGGEGKEFENGVYYYSWGGIINYNPLDQGLNNLDPLHTAMVALSLLFTKERFQNDGLVGRYSMHLGKVIRSDYSMDHLDAINQTAGVVTSDADPVQLFVDHVARLKSKGL

SEQ ID NO: 27 - DNA, 882 bp, synthetic construct
  source 1..882: mol_type = other DNA; note = AncLip8
atgtctaccagcacgactttaaaatatccagttgtactcgttcatgggctattcggatttgacaaaatcgccgggatatatccgtatttttatggcatcaaagaggctcttgaaaaagcgggagccacggtattcacagccagtatttctgcagtgaactctaatgaagtgagaggagaacagctgctggcatttgttaaagatgtgctgaaaaaaacaggggctgaaaaggtgaatctgatcggacactcgcaaggtccgcttgcttgcaggtacgtggcagcaacacatcccgaacttgtagctagtgttacaagcgtaaacggcgtcaattacggcagtgagtttgcggaccttgtccgctccgcattaaagccgggtagcttacctgaagcgattgcaaacaccgtcatgaatgccttcggtcaatttttgtctgccatttcaggaaatccgcagcttccgcaagactcgatcgcagcactcgatgcactgactacagagggcgtggcgaaatttaacgcgaagtatcctcaaggactaccagcgacatggggcggtgaaggcaaggaatttgacaatggagtttattactacagctggtcaggtattattaactataaccctctgaatcaggggctcaataaccttgatccatcccacatcgcgatggttgcttgttcccttttgttcacgaaggagcggtttcaaaatgatggcttggtaggccgatacgcttcacatttaggcaaagtcatcagatctgattattccatggatcatttggatgccataaatcagacggctggagtcgtcagctcagacgctgatccgattaaaatttatgttgaacatattgcgcgtctcaaatcaaaaggctta

SEQ ID NO: 28 - protein, 294 aa, synthetic construct
  source 1..294: note = AncLip8
MSTSTTLKYPVVLVHGLFGFDKIAGIYPYFYGIKEALEKAGATVFTASISAVNSNEVRGEQLLAFVKDVLKKTGAEKVNLIGHSQGPLACRYVAATHPELVASVTSVNGVNYGSEFADLVRSALKPGSLPEAIANTVMNAFGQFLSAISGNPQLPQDSIAALDALTTEGVAKFNAKYPQGLPATWGGEGKEFDNGVYYYSWSGIINYNPLNQGLNNLDPSHIAMVACSLLFTKERFQNDGLVGRYASHLGKVIRSDYSMDHLDAINQTAGVVSSDADPIKIYVEHIARLKSKGL

SEQ ID NO: 29 - DNA, 882 bp, synthetic construct
  source 1..882: mol_type = other DNA; note = AncLip9
atgaaaagtaatacacagacgaagtatccgatcgttctcgtgcacgggctttttgggtttgataaaatcgcgggctacccttattttttcggcattgcagaagctttaagaaagcaaggagcacaggtattcacagcttccgtcagtgccgtgaacagcacagaagttcggggagagcagttattggctcaagtaaaggaaattttaaaaaaaactggtgccgaaaaagtgaacctgatcgggcattctcagggtgcgccgacttgcaggtacgttgcggctgttcatccggagctggtggcatcagttacgtccgtaaacggtgtaaatcatggctcggagattgctgatttgcttcgaaaggtgctttctccaggttcattagccgaagcagttgccgctgcgattgtcaatgcatttggaaattttatttccttactaagtggcaacccgcagctgcctcaggacgcaatcggcgcattggattcgttgacgaccgaaggtgtagctgaatttaatcaaaaatatccccaaggtctcccaaaaacgtggggaggcgagggagctgagtttgaagtgaacggtgtctattattacagctggagcgggataataaaaaacggcctattaaatgaaggcctgaataccctggatccgtctcacgccctccttgcagtgcttagcaaattctttacaaaagaagcggaacaaaatgacggacttgtcggacgttactcatctcatctcggaaaagtcattcgcagcgattatcaaatggaccaccttgatgccatcaatcaaatggcgggaattcattcaacaaatgttgaccctgtcaacctttatgttgagcatgcagcgagactgaagtcaaaaggcctg

SEQ ID NO: 30 - protein, 294 aa, synthetic construct
  source 1..294: note = AncLip9
MKSNTQTKYPIVLVHGLFGFDKIAGYPYFFGIAEALRKQGAQVFTASVSAVNSTEVRGEQLLAQVKEILKKTGAEKVNLIGHSQGAPTCRYVAAVHPELVASVTSVNGVNHGSEIADLLRKVLSPGSLAEAVAAAIVNAFGNFISLLSGNPQLPQDAIGALDSLTTEGVAEFNQKYPQGLPKTWGGEGAEFEVNGVYYYSWSGIIKNGLLNEGLNTLDPSHALLAVLSKFFTKEAEQNDGLVGRYSSHLGKVIRSDYQMDHLDAINQMAGIHSTNVDPVNLYVEHAARLKSKGL

SEQ ID NO: 31 - DNA, 879 bp, synthetic construct
  source 1..879: mol_type = other DNA; note = AncLip10
atgaaaacgaatacgactaccaaatacccgattgttctagttcacggcttgttcggctttgataaaatcgcaggctatccttatttctttggaattaaggaagcattagaaaaagcaggtgcacaggtttttacggctagtgtttctgctgttaacagcaatgaagtgcggggagaacaactgctcgaacaggtgaaggagattctgaaaaaaaccggggctgagaaggtgaaccttataggccattcgcaaggcgccttaacctgcaggtatgtcgcagccattcatccggaacttgtagcctctgtcacgtccgtaaacggagtgaatcatggttcagaaatcgctgatttgttgagaaaagcgcttacaccaggtagtttaccagaagccgtggcggcggctgtcgtatccgcctttggcaattttatttcacttttatctggaaaccctcagctgcctcaagatgcgattgccgcgttagacgcgctgactacagaaggcgttgctgaatttaaccaaaaatatccgcaggggctgccgaaaacatggggcggcgaaggagcagaggttgtcaatggtgtatattattacagctggtcaggcattatcaaaaacgggcttttgaatcagggactcaatacacttgaccccacacatgcggcaatgagagtgctgagcaaatttttcacaaaagaagcggagcaaaatgacggtcttgtcgggcgttactcaagccacctcggaaaggtaatacgatctgattattccatggaccacttagatgcaatcaatcaaatggctggaatcgtcagcacaaacgttgatccggtaaagctctacgtggagcatgcagcgcgccttaagtcgaaaggactg

SEQ ID NO: 32 - protein, 293 aa, synthetic construct
  source 1..293: note = AncLip10
MKTNTTTKYPIVLVHGLFGFDKIAGYPYFFGIKEALEKAGAQVFTASVSAVNSNEVRGEQLLEQVKEILKKTGAEKVNLIGHSQGALTCRYVAAIHPELVASVTSVNGVNHGSEIADLLRKALTPGSLPEAVAAAVVSAFGNFISLLSGNPQLPQDAIAALDALTTEGVAEFNQKYPQGLPKTWGGEGAEVVNGVYYYSWSGIIKNGLLNQGLNTLDPTHAAMRVLSKFFTKEAEQNDGLVGRYSSHLGKVIRSDYSMDHLDAINQMAGIVSTNVDPVKLYVEHAARLKSKGL

SEQ ID NO: 33 - DNA, 879 bp, synthetic construct
  source 1..879: mol_type = other DNA; note = AncLip11
atgaaaacaaacacaacgacaaagtacccgattgttctcgttcatggattattcggttttgataaaatagccggctatccttattttttcggaatcaaagaagcgcttgaaaaagcaggggcacaagtgtttacggcttctgtttctgcggtaaactcgaatgaagtaagaggagagcagttgcttgagtttgtcaaagagattttgaaaaaaacgggtgccaaaaaggtgaacctgatcggccacagccaaggcccgctggcatgccgttacgtggctgcgatgcaccccgagcttgtcgcttccgtcacaagcgtgaatggcgtaaatcatggcagtgaaatcgcagatttggtccgaaaagcgctcaccccaggaagccttcctgaagccgttgcgaacgctgttgtaagtgctttcggcaattttatttcgcttctgtccggaaatccgcagctgcctcaggatgcgattgcggctttagacgcattaaccactgaaggcgtggccgaatttaatgcaaaatatccgcaagggttgccaaagacatggggaggagagggtaaggaagtggtcaacggtgtgtattattactcatggggcggcatcattaaaaacgggattttaaatcaagggctgaacacgcttgatccgactcatattgcaatgagagtgctgtctaaattttttacaaaagaagcagaacaaaatgacggactcgtcggccgctacagcatgcatttaggaaaagtaataaggtctgattattcaatggatcatttagacgccatcaatcagactgcaggtgttgtctcaacaaatgttgaccctgttaagctgtatgttgatcacgctgcccggctaaaatcaaagggactc

SEQ ID NO: 34 - protein, 293 aa, synthetic construct
  source 1..293: note = AncLip11
MKTNTTTKYPIVLVHGLFGFDKIAGYPYFFGIKEALEKAGAQVFTASVSAVNSNEVRGEQLLEFVKEILKKTGAKKVNLIGHSQGPLACRYVAAMHPELVASVTSVNGVNHGSEIADLVRKALTPGSLPEAVANAVVSAFGNFISLLSGNPQLPQDAIAALDALTTEGVAEFNAKYPQGLPKTWGGEGKEVVNGVYYYSWGGIIKNGILNQGLNTLDPTHIAMRVLSKFFTKEAEQNDGLVGRYSMHLGKVIRSDYSMDHLDAINQTAGVVSTNVDPVKLYVDHAARLKSKGL

SEQ ID NO: 35 - DNA, 882 bp, synthetic construct
  source 1..882: mol_type = other DNA; note = AncLip12
atgagtacaaacacgacgctgaaatatccgattgtgcttgttcacggtctgttcggttttgataaaatcgctggaatttatccttatttttatggcattaaagaagcccttgaaaaagcgggcgcaactgtttttgtcgcgacgatttctgctgtaaacagcaatgaagtgagaggagaacaattattagaattcgtgaaagaggtacttgctaaaacaggcgccaaaaaagtaaatttgatcggacactcccagggcccacttgcgtgccgctatgtcgctgcaactcacccggagctcatagcctctgtcacctcagtgaacggcgtcaatcatggttcagaaatcgcagacctggtaaggtcggcgctgacacctggttccctgccggaagccatagcgaatacagtcatgtcagcattcggacaatttttatcactgctcagtggaaatccgcagcttcctcaggattccattgaagctttggacgcattgacgacagagggggtggcaaagtttaatgcgaagtacccgcaaggactcccaagcacatggggaggcgaaggcaaggaatttgacaacggagtatattattacagctggggcgggatcatcaattacaaccccctgaatcaggggttaaacaaccttgatccgctgcatattgcaatggttgccttgagtctattgtttacaaaggagcgttttcaaaatgatgggcttgtcggcagatactcaatgcatttaggaaaagtcattcgctctgactatagcatggatcatgttgatgcgattaatcaaaccgcaggtgttgtttcttcggatgctgatcctgttaagctttatgtggaccatatcgcccggttaaaaagcaaagggttg

SEQ ID NO: 36 - protein, 294 aa, synthetic construct
  source 1..294: note = AncLip12
MSTNTTLKYPIVLVHGLFGFDKIAGIYPYFYGIKEALEKAGATVFVATISAVNSNEVRGEQLLEFVKEVLAKTGAKKVNLIGHSQGPLACRYVAATHPELIASVTSVNGVNHGSEIADLVRSALTPGSLPEAIANTVMSAFGQFLSLLSGNPQLPQDSIEALDALTTEGVAKFNAKYPQGLPSTWGGEGKEFDNGVYYYSWGGIINYNPLNQGLNNLDPLHIAMVALSLLFTKERFQNDGLVGRYSMHLGKVIRSDYSMDHVDAINQTAGVVSSDADPVKLYVDHIARLKSKGL

SEQ ID NO: 37 - DNA, 879 bp, synthetic construct
  source 1..879: mol_type = other DNA; note = AncLip13
atgaaaacgtccacaaagacgaagtacccgattgtcctcgtccacggactcttcggttttgatagaataatgggctatccgtatttttttggcatcaaagaggcactgaggaaagctggggcgcaagtgtttacggcttcaatatccgctgtaaactcaaatgaagtgagaggagaacaattattggcccaggtgaaagaaatcttgaagaaaaccggggccgaaaaagtgaacctcatcggccattctcaaggagcgccgacatgccgttatgtcgctgctgttcatccggagctggtggcatctgttaccagtgtcaacggagtcaatcatgggtcagaaattgctgacctgcttcgaagcgcgctgactcccggcagcctggttgaagcggttgcctcagcagttgtcaatgcattcgggaagtttatttctctgctctcggggaatccgcagcttcctcaggatgcgattgcagcgcttgattcattaacaacagaaggtgtggctgaatttaacaaaaaataccctcaaggtcttccaaaaacatggggaggtgaaggagcagaagtagtgaatggcgtatattattacagctggagcggcattattaaatccaacatcttagatcagggcttaaatgccttagacccaactcacattgtgcttgtagcattgtctaaatttttcacgaaagaggcggatcaaaacgacggcctagtcggacgctattcttcgcatttaggaaaagttatccgcagcgattatcagatggatcatttggatgcgatcaatcaaatggccggtgttcacagcacaaatgttgaccctgttagtctttacgtagagcatgcagcccggctgaagtcaaaaggcctt

SEQ ID NO: 38 - protein, 293 aa, synthetic construct
  source 1..293: note = AncLip13
MKTSTKTKYPIVLVHGLFGFDRIMGYPYFFGIKEALRKAGAQVFTASISAVNSNEVRGEQLLAQVKEILKKTGAEKVNLIGHSQGAPTCRYVAAVHPELVASVTSVNGVNHGSEIADLLRSALTPGSLVEAVASAVVNAFGKFISLLSGNPQLPQDAIAALDSLTTEGVAEFNKKYPQGLPKTWGGEGAEVVNGVYYYSWSGIIKSNILDQGLNALDPTHIVLVALSKFFTKEADQNDGLVGRYSSHLGKVIRSDYQMDHLDAINQMAGVHSTNVDPVSLYVEHAARLKSKGL

SEQ ID NO: 39 - DNA, 882 bp, synthetic construct
  source 1..882: mol_type = other DNA; note = AncLip14
atgaaaacttctacacaaacaaaatatccgattgtccttgtgcacggcctgttcggatttgataaaatcgccggctatccttattttttcggcatcaaagaagcgcttgaaagagccggagcaaaagtatttacggcttcaatatctgcgacaaattcaactgaggtgagaggagaacagcttttagcacaggtgaaacaaattttaaaaaaaacaggtgctgaaaaggtaaacctgatcggccattctcaaggcgcactcacatgccgctacgtagccgcagtccatcctgagcttgtagcctcggtcacctccgtgaatggtgtaaatcatggaagtgaaattgctgacttgctccgtaaagtgcttacccccggttctctcgcggaagctgttgctgcaaccgttgtgaacgcttttgggaacttcatcagcttactaagcggaaatccgcagctgcctcaggatgcgattgcggcgctggactccctgacaacagaaggcgtggcagaatttaatcaaaaatacccgcaagggttgccaacgacttggggcggcgaaggaaaggagctggcatctaacggtgtttactattattcatggagcggaattataaaaggcaatttgttaaaccaggggttgaatacgctcgatccatcacatgcagcacttgcggttttatcgaaattttttacaaaggaaaaagagcaaaacgacggtcttgtcggtcgatattcctcacaccttggaaaagtcatcaggagtgattatccgatggatcatttagacgctgtcaatcagacggccgggattcacagcagcaatgttgatccggttaagctgtacgttgagcatgccgcccggttgaagtcaaaggggctg

SEQ ID NO: 40 - protein, 294 aa, synthetic construct
  source 1..294: note = AncLip14
MKTSTQTKYPIVLVHGLFGFDKIAGYPYFFGIKEALERAGAKVFTASISATNSTEVRGEQLLAQVKQILKKTGAEKVNLIGHSQGALTCRYVAAVHPELVASVTSVNGVNHGSEIADLLRKVLTPGSLAEAVAATVVNAFGNFISLLSGNPQLPQDAIAALDSLTTEGVAEFNQKYPQGLPTTWGGEGKELASNGVYYYSWSGIIKGNLLNQGLNTLDPSHAALAVLSKFFTKEKEQNDGLVGRYSSHLGKVIRSDYPMDHLDAVNQTAGIHSSNVDPVKLYVEHAARLKSKGL

SEQ ID NO: 41 - DNA, 879 bp, synthetic construct
  source 1..879: mol_type = other DNA; note = AncLip15
atgagcacaaacacaaaaacgaaatacccgattgttctcgtacacgggctgttcggcttcgataagatcgcgggctatccctatttttatggaatcgctgaggcgttaagaaagcagggcgcgactgtttttacagctagtatctccgctgccaacagcaccgaggttaggggagaacagctactggcacaaattaaagaaattttaaaaaaaacaggagcacaaaaagtcaatctgattggccattctcaaggtgcacctacgtgcagatatgtggcggctgtacatcctgaattggtggcttctgtcacctccgttaacggtgtgaatcacggcagtgaaatagccgatttattacgaaaggtattaagtccaggtagccttgcagaagcagtagctgcggcccttgtaaacgcttttggctcatttatttcattattgtcgggaaatccgcaattgccgcaggatgcgattgcagccttgaattcgctgactactgagggggtcgccgaatttaacgcaaaatatcctcaggggttaccgacaacatggggaggcgaaggagcggaagaagtgaacggcgtttattattacagctggtcaggtataatcaaaggcaatcttcttgatcaagggctgaatacgctggatccatctcatgcgcttctcgcagcgctcagcaagtttttcacgaaggaagcagagcagaatgacggtctcgtcggccgttactcttcacacctgggaaaagtgattcgctctgattatccgatggatcatcttgacgccatcaatcaaatggcgggggtgcattcaacaaatgttgaccctgtcaacctatacgtcgaccatgctgcccggctgaaatcaaaaggactt

SEQ ID NO: 42 - protein, 293 aa, synthetic construct
  source 1..293: note = AncLip15
MSTNTKTKYPIVLVHGLFGFDKIAGYPYFYGIAEALRKQGATVFTASISAANSTEVRGEQLLAQIKEILKKTGAQKVNLIGHSQGAPTCRYVAAVHPELVASVTSVNGVNHGSEIADLLRKVLSPGSLAEAVAAALVNAFGSFISLLSGNPQLPQDAIAALNSLTTEGVAEFNAKYPQGLPTTWGGEGAEEVNGVYYYSWSGIIKGNLLDQGLNTLDPSHALLAALSKFFTKEAEQNDGLVGRYSSHLGKVIRSDYPMDHLDAINQMAGVHSTNVDPVNLYVDHAARLKSKGL

SEQ ID NO: 43 - DNA, 879 bp, synthetic construct
  source 1..879: mol_type = other DNA; note = AncLip16
atgtctacttcagcccagacgaaatacccgattgtcctagttcacggtttgttcggctttgatcggatagccggctacccatattggtatggcatcaaagaagcattaagaaaggcgggcgcgcaggtatatgtggctcaggtcagcgctgttcattcaaatgaagtacgcggtgaacaactgcttgagcaaattgaagaaatcctcagacaaacgggggcgcaaaaagtaaacctcattggccacagccaaggcgccttaaccgcacgttatgctgcagctgtccgtcctgagctggttgcaagcgtaacaagtgtttctggacctaaccatggctcggagcttgccgacctgctgcgcaaaaaattaccacccggttctcttccggaggctcttgctgcagccgtgatgaatgcgctcgggtcctttatttcactgttatctggggggccgcagcttccacaggatgccttagctgcacttcaagcgttgacgacagaaggtgtggccgcatttaatcaaaagtacccgcaaggactacctgaaacatggggaggagaaggcgcagaagtggtgaacggcgttcgctattattcgtggagcggcaccattcagccgaacattacagatcaggggctgaatgcactggacccgtcacacgcgctttgccgtgctctgtcccgatgttttactagagaagccggacaaaatgacggaatggtcggacggttcagctctcatttgggaaaagtgatcagatccgattacccgatggatcatttagatacaatcaatcagctggcaggtcttgttggacataacgtcgaccctgtggcgttgtatgtagagcatgcggctaggctgaagagtgcgggcctc

SEQ ID NO: 44 - protein, 293 aa, synthetic construct
  source 1..293: note = AncLip16
MSTSAQTKYPIVLVHGLFGFDRIAGYPYWYGIKEALRKAGAQVYVAQVSAVHSNEVRGEQLLEQIEEILRQTGAQKVNLIGHSQGALTARYAAAVRPELVASVTSVSGPNHGSELADLLRKKLPPGSLPEALAAAVMNALGSFISLLSGGPQLPQDALAALQALTTEGVAAFNQKYPQGLPETWGGEGAEVVNGVRYYSWSGTIQPNITDQGLNALDPSHALCRALSRCFTREAGQNDGMVGRFSSHLGKVIRSDYPMDHLDTINQLAGLVGHNVDPVALYVEHAARLKSAGL

SEQ ID NO: 45 - DNA, 879 bp, synthetic construct
  source 1..879: mol_type = other DNA; note = uncultured bacterium-derived sequence
atgtcggcttctagcctgaaatttccgatcgtgctcgttcacggcctgttaggttttgataaaatcggcggaatctatccttatttttacggcattaaagaggcgcttgaaaaagcgggagcgaaggtttatattgcgacactttctgctttgaacagcaatgaacttcgcggagaacagttgttggaatttgtcagaaaagttcaggcagaaacaggcgcggcaaaagtgaatcttattggacactcacaaggcccgctggcatgccgctatgtggcggccactcatccggagctgattgcatctgtcacgtcggtaaacggcgtcaatcatgggagtgaagtggctgatcttgtaagattggctctgacaccgggacgactccctgaatccatagccaatgcagcgatgtcagcattcggacagttactctcggcattggccgggtcaccccgtcttccacagtcaggaattgaagcattagaagctttaacgtctgaaggagttgccgcctttaacaataaatatccgcaaggactgcctgctgaatggggcggtgagggcaaagaattggtaaacggtgtatattattactcttggagcggtgtgattgattataaccctcttcatcagggggcaaacaacttagacccgcttcatgtcgcaatgctggctttctccatcctgtttactaatgagcgttttcaaaatgacgggcttgtcggccggtactcctcacacctaggaaaagtcattgggagtgattacagcatggatcatgttgatgcgatcaatcaattagccggtgttgtcgctaataacaccgacccagttcaattattcgtggagcatgtggcgaggctgaagagcaagggcctc

SEQ ID NO: 46 - protein, 293 aa, unidentified
  source 1..293: note = uncultured bacterium-derived sequence
MSASSLKFPIVLVHGLLGFDKIGGIYPYFYGIKEALEKAGAKVYIATLSALNSNELRGEQLLEFVRKVQAETGAAKVNLIGHSQGPLACRYVAATHPELIASVTSVNGVNHGSEVADLVRLALTPGRLPESIANAAMSAFGQLLSALAGSPRLPQSGIEALEALTSEGVAAFNNKYPQGLPAEWGGEGKELVNGVYYYSWSGVIDYNPLHQGANNLDPLHVAMLAFSILFTNERFQNDGLVGRYSSHLGKVIGSDYSMDHVDAINQLAGVVANNTDPVQLFVEHVARLKSKGL

SEQ ID NO: 47 - DNA, 807 bp, synthetic construct
  source 1..807: mol_type = other DNA; note = Thermomyces lanuginosus-derived sequence
gaagtgagccaagatttatttaaccagtttaacctgtttgcgcaatattctgcagcggcttattgcggaaaaaataacgatgccccggcaggaacaaatatcacatgcacaggcaacgcttgtccggaagttgaaaaagcggatgctacatttctttactcatttgaagatagcggcgtgggagatgtcacaggctttctggcccttgataacacaaacaaactgatcgtgctgtcatttagaggaagccgctctatcgaaaactggatcggcaaccttaactttgatctgaaagaaatcaacgatatctgctcaggctgtagaggacatgatggctttacatcaagctggagaagcgtcgcggatacattacgccagaaagttgaagatgctgtgagagaacatccggattatcgcgttgtgtttacaggacattctctgggcggagcccttgcaacagttgctggagctgatctgagaggcaacggatacgatatcgatgtcttttcatacggagctccgagagttggcaaccgcgcctttgcagaatttcttacagtgcaaacaggcggaacactgtaccgcatcacacatacaaacgatattgtcccgagactgccgccgcgcgaatttggatattctcattcttcaccggaatattggatcaaatcaggcacacttgtcccggttacacgcaacgatatcgttaaaatcgaaggaatcgatgccacaggcggaaataaccagccgaacatcccggatattccggcacatttatggtattttggactgattggcacatgtctt

SEQ ID NO: 48 - protein, 269 aa, Thermomyces lanuginosus [sequence omitted]

SEQ ID NO: 49 - DNA, 99 bp, synthetic construct
  source 1..99: mol_type = other DNA; note = Bacillus subtilis-derived sequence
atgtttgcaaaacgattcaaaacctctttactgccgttattcgctggatttttattgctgtttcatttggttctggcaggaccggcggctgcgagtgct

SEQ ID NO: 50 - protein, 33 aa, Bacillus subtilis
MFAKRFKTSLLPLFAGFLLLFHLVLAGPAAASA